European Patent Specification EP 3 717 636 B1, published March 8, 2023. Title: ADENO-ASSOCIATED VIRUS VARIANT CAPSIDS AND USE FOR INHIBITING ANGIOGENESIS. Applicant: 4D Molecular Therapeutics Inc. The sequence listing filed with the application follows.

SEQUENCE LISTING (77 sequences)

SEQ ID NO: 1 - protein, 736 aa, Adeno-associated virus 1
MAADGYLPDWLEDNLSEGIREWWDLKPGAPKPKANQQKQDDGRGLVLPGYKYLGPFNGLDKGEPVNAADAAALEHDKAYDQQLKAGDNPYLRYNHADAEFQERLQEDTSFGGNLGRAVFQAKKRVLEPLGLVEEGAKTAPGKKRPVEQSPQEPDSSSGIGKTGQQPAKKRLNFGQTGDSESVPDPQPLGEPPATPAAVGPTTMASGGGAPMADNNEGADGVGNASGNWHCDSTWLGDRVITTSTRTWALPTYNNHLYKQISSASTGASNDNHYFGYSTPWGYFDFNRFHCHFSPRDWQRLINNNWGFRPKRLNFKLFNIQVKEVTTNDGVTTIANNLTSTVQVFSDSEYQLPYVLGSAHQGCLPPFPADVFMIPQYGYLTLNNGSQAVGRSSFYCLEYFPSQMLRTGNNFTFSYTFEEVPFHSSYAHSQSLDRLMNPLIDQYLYYLNRTQNQSGSAQNKDLLFSRGSPAGMSVQPKNWLPGPCYRQQRVSKTKTDNNNSNFTWTGASKYNLNGRESIINPGTAMASHKDDEDKFFPMSGVMIFGKESAGASNTALDNVMITDEEEIKATNPVATERFGTVAVNFQSSSTDPATGDVHAMGALPGMVWQDRDVYLQGPIWAKIPHTDGHFHPSPLMGGFGLKNPPPQILIKNTPVPANPPAEFSATKFASFITQYSTGQVSVEIEWELQKENSKRWNPEVQYTSNYAKSANVDFTVDNNGLYTEPRPIGTRYLTRPL

SEQ ID NO: 2 - protein, 735 aa, Adeno-associated virus 2 [sequence omitted]

SEQ ID NO: 3 - protein, 736 aa, Adeno-associated virus 3A
MAADGYLPDWLEDNLSEGIREWWALKPGVPQPKANQQHQDNRRGLVLPGYKYLGPGNGLDKGEPVNEADAAALEHDKAYDQQLKAGDNPYLKYNHADAEFQERLQEDTSFGGNLGRAVFQAKKRILEPLGLVEEAAKTAPGKKGAVDQSPQEPDSSSGVGKSGKQPARKRLNFGQTGDSESVPDPQPLGEPPAAPTSLGSNTMASGGGAPMADNNEGADGVGNSSGNWHCDSQWLGDRVITTSTRTWALPTYNNHLYKQISSQSGASNDNHYFGYSTPWGYFDFNRFHCHFSPRDWQRLINNNWGFRPKKLSFKLFNIQVRGVTQNDGTTTIANNLTSTVQVFTDSEYQLPYVLGSAHQGCLPPFPADVFMVPQYGYLTLNNGSQAVGRSSFYCLEYFPSQMLRTGNNFQFSYTFEDVPFHSSYAHSQSLDRLMNPLIDQYLYYLNRTQGTTSGTTNQSRLLFSQAGPQSMSLQARNWLPGPCYRQQRLSKTANDNNNSNFPWTAASKYHLNGRDSLVNPGPAMASHKDDEEKFFPMHGNLIFGKEGTTASNAELDNVMITDEEEIRTTNPVATEQYGTVANNLQSSNTAPTTGTVNHQGALPGMVWQDRDVYLQGPIWAKIPHTDGHFHPSPLMGGFGLKHPPPQIMIKNTPVPANPPTTFSPAKFASFITQYSTGQVSVEIEWELQKENSKRWNPEIQYTSNYNKSVNVDFTVDTNGVYSEPRPIGTRYLTRNL

SEQ ID NO: 4 - protein, 736 aa, Adeno-associated virus 3B
MAADGYLPDWLEDNLSEGIREWWALKPGVPQPKANQQHQDNRRGLVLPGYKYLGPGNGLDKGEPVNEADAAALEHDKAYDQQLKAGDNPYLKYNHADAEFQERLQEDTSFGGNLGRAVFQAKKRILEPLGLVEEAAKTAPGKKRPVDQSPQEPDSSSGVGKSGKQPARKRLNFGQTGDSESVPDPQPLGEPPAAPTSLGSNTMASGGGAPMADNNEGADGVGNSSGNWHCDSQWLGDRVITTSTRTWALPTYNNHLYKQISSQSGASNDNHYFGYSTPWGYFDFNRFHCHFSPRDWQRLINNNWGFRPKKLSFKLFNIQVKEVTQNDGTTTIANNLTSTVQVFTDSEYQLPYVLGSAHQGCLPPFPADVFMVPQYGYLTLNNGSQAVGRSSFYCLEYFPSQMLRTGNNFQFSYTFEDVPFHSSYAHSQSLDRLMNPLIDQYLYYLNRTQGTTSGTTNQSRLLFSQAGPQSMSLQARNWLPGPCYRQQRLSKTANDNNNSNFPWTAASKYHLNGRDSLVNPGPAMASHKDDEEKFFPMHGNLIFGKEGTTASNAELDNVMITDEEEIRTTNPVATEQYGTVANNLQSSNTAPTTRTVNDQGALPGMVWQDRDVYLQGPIWAKIPHTDGHFHPSPLMGGFGLKHPPPQIMIKNTPVPANPPTTFSPAKFASFITQYSTGQVSVEIEWELQKENSKRWNPEIQYTSNYNKSVNVDFTVDTNGVYSEPRPIGTRYLTRNL

SEQ ID NO: 5 - protein, 734 aa, Adeno-associated virus 4
MTDGYLPDWLEDNLSEGVREWWALQPGAPKPKANQQHQDNARGLVLPGYKYLGPGNGLDKGEPVNAADAAALEHDKAYDQQLKAGDNPYLKYNHADAEFQQRLQGDTSFGGNLGRAVFQAKKRVLEPLGLVEQAGETAPGKKRPLIESPQQPDSSTGIGKKGKQPAKKKLVFEDETGAGDGPPEGSTSGAMSDDSEMRAAAGGAAVEGGQGADGVGNASGDWHCDSTWSEGHVTTTSTRTWVLPTYNNHLYKRLGESLQSNTYNGFSTPWGYFDFNRFHCHFSPRDWQRLINNNWGMRPKAMRVKIFNIQVKEVTTSNGETTVANNLTSTVQIFADSSYELPYVMDAGQEGSLPPFPNDVFMVPQYGYCGLVTGNTSQQQTDRNAFYCLEYFPSQMLRTGNNFEITYSFEKVPFHSMYAHSQSLDRLMNPLIDQYLWGLQSTTTGTTLNAGTATTNFTKLRPTNFSNFKKNWLPGPSIKQQGFSKTANQNYKIPATGSDSLIKYETHSTLDGRWSALTPGPPMATAGPADSKFSNSQLIFAGPKQNGNTATVPGTLIFTSEEELAATNATDTDMWGNLPGGDQSNSNLPTVDRLTALGAVPGMVWQNRDIYYQGPIWAKIPHTDGHFHPSPLIGGFGLKHPPPQIFIKNTPVPANPATTFSSTPVNSFITQYSTGQVSVQIDWEIQKERSKRWNPEVQFTSNYGQQNSLLWAPDAAGKYTEPRAIGTRYLTHHL

SEQ ID NO: 6 - protein, 724 aa, Adeno-associated virus 5
MSFVDHPPDWLEEVGEGLREFLGLEAGPPKPKPNQQHQDQARGLVLPGYNYLGPGNGLDRGEPVNRADEVAREHDISYNEQLEAGDNPYLKYNHADAEFQEKLADDTSFGGNLGKAVFQAKKRVLEPFGLVEEGAKTAPTGKRIDDHFPKRKKARTEEDSKPSTSSDAEAGPSGSQQLQIPAQPASSLGADTMSAGGGGPLGDNNQGADGVGNASGDWHCDSTWMGDRVVTKSTRTWVLPSYNNHQYREIKSGSVDGSNANAYFGYSTPWGYFDFNRFHSHWSPRDWQRLINNYWGFRPRSLRVKIFNIQVKEVTVQDSTTTIANNLTSTVQVFTDDDYQLPYVVGNGTEGCLPAFPPQVFTLPQYGYATLNRDNTENPTERSSFFCLEYFPSKMLRTGNNFEFTYNFEEVPFHSSFAPSQNLFKLANPLVDQYLYRFVSTNNTGGVQFNKNLAGRYANTYKNWFPGPMGRTQGWNLGSGVNRASVSAFATTNRMELEGASYQVPPQPNGMTNNLQGSNTYALENTMIFNSQPANPGTTATYLEGNMLITSESETQPVNRVAYNVGGQMATNNQSSTTAPATGTYNLQEIVPGSVWMERDVYLQGPIWAKIPETGAHFHPSPAMGGFGLKHPPPMMLIKNTPVPGNITSFSDVPVSSFITQYSTGQVTVEMEWELKKENSKRWNPEIQYTNNYNDPQFVDFAPDSTGEYRTTRPIGTRYLTRPL

SEQ ID NO: 7 - protein, 736 aa, Adeno-associated virus 6
MAADGYLPDWLEDNLSEGIREWWDLKPGAPKPKANQQKQDDGRGLVLPGYKYLGPFNGLDKGEPVNAADAAALEHDKAYDQQLKAGDNPYLRYNHADAEFQERLQEDTSFGGNLGRAVFQAKKRVLEPFGLVEEGAKTAPGKKRPVEQSPQEPDSSSGIGKTGQQPAKKRLNFGQTGDSESVPDPQPLGEPPATPAAVGPTTMASGGGAPMADNNEGADGVGNASGNWHCDSTWLGDRVITTSTRTWALPTYNNHLYKQISSASTGASNDNHYFGYSTPWGYFDFNRFHCHFSPRDWQRLINNNWGFRPKRLNFKLFNIQVKEVTTNDGVTTIANNLTSTVQVFSDSEYQLPYVLGSAHQGCLPPFPADVFMIPQYGYLTLNNGSQAVGRSSFYCLEYFPSQMLRTGNNFTFSYTFEDVPFHSSYAHSQSLDRLMNPLIDQYLYYLNRTQNQSGSAQNKDLLFSRGSPAGMSVQPKNWLPGPCYRQQRVSKTKTDNNNSNFTWTGASKYNLNGRESIINPGTAMASHKDDKDKFFPMSGVMIFGKESAGASNTALDNVMITDEEEIKATNPVATERFGTVAVNLQSSSTDPATGDVHVMGALPGMVWQDRDVYLQGPIWAKIPHTDGHFHPSPLMGGFGLKHPPPQILIKNTPVPANPPAEFSATKFASFITQYSTGQVSVEIEWELQKENSKRWNPEVQYTSNYAKSANVDFTVDNNGLYTEPRPIGTRYLTRPL

SEQ ID NO: 8 - protein, 737 aa, Adeno-associated virus 7
MAADGYLPDWLEDNLSEGIREWWDLKPGAPKPKANQQKQDNGRGLVLPGYKYLGPFNGLDKGEPVNAADAAALEHDKAYDQQLKAGDNPYLRYNHADAEFQERLQEDTSFGGNLGRAVFQAKKRVLEPLGLVEEGAKTAPAKKRPVEPSPQRSPDSSTGIGKKGQQPARKRLNFGQTGDSESVPDPQPLGEPPAAPSSVGSGTVAAGGGAPMADNNEGADGVGNASGNWHCDSTWLGDRVITTSTRTWALPTYNNHLYKQISSETAGSTNDNTYFGYSTPWGYFDFNRFHCHFSPRDWQRLINNNWGFRPKKLRFKLFNIQVKEVTTNDGVTTIANNLTSTIQVFSDSEYQLPYVLGSAHQGCLPPFPADVFMIPQYGYLTLNNGSQSVGRSSFYCLEYFPSQMLRTGNNFEFSYSFEDVPFHSSYAHSQSLDRLMNPLIDQYLYYLARTQSNPGGTAGNRELQFYQGGPSTMAEQAKNWLPGPCFRQQRVSKTLDQNNNSNFAWTGATKYHLNGRNSLVNPGVAMATHKDDEDRFFPSSGVLIFGKTGATNKTTLENVLMTNEEEIRPTNPVATEEYGIVSSNLQAANTAAQTQVVNNQGALPGMVWQNRDVYLQGPIWAKIPHTDGNFHPSPLMGGFGLKHPPPQILIKNTPVPANPPEVFTPAKFASFITQYSTGQVSVEIEWELQKENSKRWNPEIQYTSNFEKQTGVDFAVDSQGVYSEPRPIGTRYLTRNL

SEQ ID NO: 9 - protein, 738 aa, Adeno-associated virus 8
MAADGYLPDWLEDNLSEGIREWWALKPGAPKPKANQQKQDDGRGLVLPGYKYLGPFNGLDKGEPVNAADAAALEHDKAYDQQLQAGDNPYLRYNHADAEFQERLQEDTSFGGNLGRAVFQAKKRVLEPLGLVEEGAKTAPGKKRPVEPSPQRSPDSSTGIGKKGQQPARKRLNFGQTGDSESVPDPQPLGEPPAAPSGVGPNTMAAGGGAPMADNNEGADGVGSSSGNWHCDSTWLGDRVITTSTRTWALPTYNNHLYKQISNGTSGGATNDNTYFGYSTPWGYFDFNRFHCHFSPRDWQRLINNNWGFRPKRLSFKLFNIQVKEVTQNEGTKTIANNLTSTIQVFTDSEYQLPYVLGSAHQGCLPPFPADVFMIPQYGYLTLNNGSQAVGRSSFYCLEYFPSQMLRTGNNFQFTYTFEDVPFHSSYAHSQSLDRLMNPLIDQYLYYLSRTQTTGGTANTQTLGFSQGGPNTMANQAKNWLPGPCYRQQRVSTTTGQNNNSNFAWTAGTKYHLNGRNSLANPGIAMATHKDDEERFFPSNGILIFGKQNAARDNADYSDVMLTSEEEIKTTNPVATEEYGIVADNLQQQNTAPQIGTVNSQGALPGMVWQNRDVYLQGPIWAKIPHTDGNFHPSPLMGGFGLKHPPPQILIKNTPVPADPPTTFNQSKLNSFITQYSTGQVSVEIEWELQKENSKRWNPEIQYTSNYYKSTSVDFAVNTEGVYSEPRPIGTRYLTRNL

SEQ ID NO: 10 - protein, 736 aa, Adeno-associated virus 9
MAADGYLPDWLEDNLSEGIREWWALKPGAPQPKANQQHQDNARGLVLPGYKYLGPGNGLDKGEPVNAADAAALEHDKAYDQQLKAGDNPYLKYNHADAEFQERLKEDTSFGGNLGRAVFQAKKRLLEPLGLVEEAAKTAPGKKRPVEQSPQEPDSSAGIGKSGAQPAKKRLNFGQTGDTESVPDPQPIGEPPAAPSGVGSLTMASGGGAPVADNNEGADGVGSSSGNWHCDSQWLGDRVITTSTRTWALPTYNNHLYKQISNSTSGGSSNDNAYFGYSTPWGYFDFNRFHCHFSPRDWQRLINNNWGFRPKRLNFKLFNIQVKEVTDNNGVKTIANNLTSTVQVFTDSDYQLPYVLGSAHEGCLPPFPADVFMIPQYGYLTLNDGSQAVGRSSFYCLEYFPSQMLRTGNNFQFSYEFENVPFHSSYAHSQSLDRLMNPLIDQYLYYLSKTINGSGQNQQTLKFSVAGPSNMAVQGRNYIPGPSYRQQRVSTTVTQNNNSEFAWPGASSWALNGRNSLMNPGPAMASHKEGEDRFFPLSGSLIFGKQGTGRDNVDADKVMITNEEEIKTTNPVATESYGQVATNHQSAQAQAQTGWVQNQGILPGMVWQDRDVYLQGPIWAKIPHTDGNFHPSPLMGGFGMKHPPPQILIKNTPVPADPPTAFNKDKLNSFITQYSTGQVSVEIEWELQKENSKRWNPEIQYTSNYYKSNNVEFAVNTEGVYSEPRPIGTRYLTRNL

SEQ ID NO: 11 - protein, 738 aa, Adeno-associated virus 10
MAADGYLPDWLEDNLSEGIREWWDLKPGAPKPKANQQKQDDGRGLVLPGYKYLGPFNGLDKGEPVNAADAAALEHDKAYDQQLKAGDNPYLRYNHADAEFQERLQEDTSFGGNLGRAVFQAKKRVLEPLGLVEEAAKTAPGKKRPVEPSPQRSPDSSTGIGKKGQQPAKKRLNFGQTGESESVPDPQPIGEPPAGPSGLGSGTMAAGGGAPMADNNEGADGVGSSSGNWHCDSTWLGDRVITTSTRTWALPTYNNHLYKQISNGTSGGSTNDNTYFGYSTPWGYFDFNRFHCHFSPRDWQRLINNNWGFRPKRLSFKLFNIQVKEVTQNEGTKTIANNLTSTIQVFTDSEYQLPYVLGSAHQGCLPPFPADVFMIPQYGYLTLNNGSQAVGRSSFYCLEYFPSQMLRTGNNFEFSYTFEDVPFHSSYAHSQSLDRLMNPLIDQYLYYLSRTQSTGGTQGTQQLLFSQAGPANMSAQAKNWLPGPCYRQQRVSTTLSQNNNSNFAWTGATKYHLNGRDSLVNPGVAMATHKDDEERFFPSSGVLMFGKQGAGRDNVDYSSVMLTSEEEIKTTNPVATEQYGVVADNLQQANTGPIVGNVNSQGALPGMVWQNRDVYLQGPIWAKIPHTDGNFHPSPLMGGFGLKHPPPQILIKNTPVPADPPTTFSQAKLASFITQYSTGQVSVEIEWELQKENSKRWNPEIQYTSNYYKSTNVDFAVNTEGTYSEPRPIGTRYLTRNL

SEQ ID NO: 12 - protein, 738 aa, Adeno-associated virus rh10
MAADGYLPDWLEDNLSEGIREWWALKPGAPKPKANQQKQDDGRGLVLPGYKYLGPFNGLDKGEPVNAADAAALEHDKAYDQQLKAGDNPYLRYNHADAEFQERLQEDTSFGGNLGRAVFQAKKRVLEPLGLVEEGAKTAPGKKRPVEPSPQRSPDSSTGIGKKGQQPAKKRLNFGQTGDSESVPDPQPIGEPPAGPSGLGSGTMAAGGGAPMADNNEGADGVGSSSGNWHCDSTWLGDGVITTSTRTWALPTYNNHLYKQISNGTSGGSTNDNTYFGYSTPWGYFDFNRFHCHFSPRDWQRLINNNWGFRPKSLNFKLFNIQVKEVTQNEGTKTIANNLTSTIQVFTDSEYQLPYVLGSAHQGCLPPFPADVFMIPQYGYLTLNNGSQAVGRSSFYCLEYFPSQMLRTGNNFEFSYQFEDVPFHSSYAHSQSLDRLMNPLIDQYLYYLSRTQSTGGTAGTQQLLFSQAGPNNMSAQAKNWLPGPCYRQQRVSTTLSQNDNSNFAWTGATKYHLNGRDSLVNPGVAMATHKDDEERFFPSSGVLMFGKQGAGKDNVDYSSVMLTSEEEIKTTNPVATEQYGVVADNLQQQNAAPIVGAVNSQGALPGMVWQNRDVYLQGPIWAKIPHTDGNFHPSPLMGGFGLKHPPPQILIKNTPVPADPPTTFSQAKLASFITQYSTGQVSVEIEWELQKENSKRWNPEIQYTSNYYKSTNVDFAVNTDGTYSEPRPIGTRYLTRNL

SEQ ID NO: 13 - protein, 7 aa, Artificial Sequence
  heterologous peptide insertion
QADTTKN

SEQ ID NO: 14 - protein, 7 aa, Artificial Sequence
  heterologous peptide insertion
ISDQTKH

SEQ ID NO: 15 - protein, 7 aa, Artificial Sequence
  heterologous peptide insertion
ASDSTKA

SEQ ID NO: 16 - protein, 7 aa, Artificial Sequence
  heterologous peptide insertion
NQDYTKT

SEQ ID NO: 17 - protein, 7 aa, Artificial Sequence
  heterologous peptide insertion
HDITKNI

SEQ ID NO: 18 - protein, 7 aa, Artificial Sequence
  heterologous peptide insertion
HPDTTKN

SEQ ID NO: 19 - protein, 7 aa, Artificial Sequence
  heterologous peptide insertion
HQDTTKN

SEQ ID NO: 20 - protein, 7 aa, Artificial Sequence
  heterologous peptide insertion
NKTTNKD

SEQ ID NO: 21 - protein, 7 aa, Artificial Sequence
  heterologous peptide insertion
ISNENEH

SEQ ID NO: 22 - protein, 7 aa, Artificial Sequence
  heterologous peptide insertion
QANANEN

SEQ ID NO: 23 - protein, 7 aa, Artificial Sequence
  heterologous peptide insertion
GKSKVID

SEQ ID NO: 24 - protein, 7 aa, Artificial Sequence
  heterologous peptide insertion
TNRTSPD

SEQ ID NO: 25 - protein, 7 aa, Artificial Sequence
  heterologous peptide insertion
PNSTHGS

SEQ ID NO: 26 - protein, 7 aa, Artificial Sequence
  heterologous peptide insertion
KDRAPST

SEQ ID NO: 27 - protein, 10 aa, Artificial Sequence
  heterologous peptide insertion
LAQADTTKNA

SEQ ID NO: 28 - protein, 10 aa, Artificial Sequence
  heterologous peptide insertion
LAISDQTKHA

SEQ ID NO: 29 - protein, 10 aa, Artificial Sequence
  heterologous peptide insertion
LGISDQTKHA

SEQ ID NO: 30 - protein, 10 aa, Artificial Sequence
  heterologous peptide insertion
LAASDSTKAA

SEQ ID NO: 31 - protein, 10 aa, Artificial Sequence
  heterologous peptide insertion
LANQDYTKTA

SEQ ID NO: 32 - protein, 10 aa, Artificial Sequence
  heterologous peptide insertion
LAHDITKNIA

SEQ ID NO: 33 - protein, 10 aa, Artificial Sequence
  heterologous peptide insertion
LAHPDTTKNA

SEQ ID NO: 34 - protein, 10 aa, Artificial Sequence
  heterologous peptide insertion
LAHQDTTKNA

SEQ ID NO: 35 - protein, 10 aa, Artificial Sequence
  heterologous peptide insertion
LANKTTNKDA

SEQ ID NO: 36 - protein, 10 aa, Artificial Sequence
  heterologous peptide insertion
LPISNENEHA

SEQ ID NO: 37 - protein, 10 aa, Artificial Sequence
  heterologous peptide insertion
LPQANANENA

SEQ ID NO: 38 - protein, 10 aa, Artificial Sequence
  heterologous peptide insertion
LAGKSKVIDA

SEQ ID NO: 39 - protein, 10 aa, Artificial Sequence
  heterologous peptide insertion
LATNRTSPDA

SEQ ID NO: 40 - protein, 10 aa, Artificial Sequence
  heterologous peptide insertion
LAPNSTHGSA

SEQ ID NO: 41 - protein, 10 aa, Artificial Sequence
  heterologous peptide insertion
LAKDRAPSTA

SEQ ID NO: 42 - protein, 745 aa, Artificial Sequence
  Variant AAV capsid
MAADGYLPDWLEDTLSEGIRQWWKLKPGPPPPKAAERHKDDSRGLVLPGYKYLGPFNGLDKGEPVNEADAAALEHDKAYDRQLDSGDNPYLKYNHADAEFQERLKEDTSFGGNLGRAVFQAKKRVLEPLGLVEEPVKTAPGKKRPVEHSPVEPDSSSGTGKAGQQPARKRLNFGQTGDADSVPDPQPLGQPPAAPSGLGTNTMATGSGAPMADNNEGADGVGNSSGNWHCDSTWMGDRVITTSTRTWALPTYNNHLYKQISSQSGASNDNHYFGYSTPWGYFDFNRFHCHFSPRDWQRLINNNWGFRPKRLNFKLFNIQVKEVTQNDGTTTIANNLTSTVQVFTDSEYQLPYVLGSAHQGCLPPFPADVFMVPQYGYLTLNNGSQAVGRSSFYCLEYFPSQMLRTGNNFTFSYTFEDVPFHSSYAHSQSLDRLMNPLIDQYLYYLSRTNTPSGTTTQSRLQFSQAGASDIRDQSRNWLPGPCYRQQRVSKTSADNNNSEYSWTGATKYHLNGRDSLVNPGPAMASHKDDEEKFFPQSGVLIFGKQGSEKTNVDIEKVMITDEEEIRTTNPVATEQYGSVSTNLQRGNLAISDQTKHARQAATADVNTQGVLPGMVWQDRDVYLQGPIWAKIPHTDGHFHPSPLMGGFGLKHPPPQILIKNTPVPANPSTTFSAAKFASFITQYSTGQVSVEIEWELQKENSKRWNPEIQYTSNYNKSVNVDFTVDTNGVYSEPRPIGTRYLTRNL

SEQ ID NO: 43 - protein, 745 aa, Artificial Sequence
  AAV capsid variant
MAADGYLPDWLEDTLSEGIRQWWKLKPGPPPPKPAERHKDDSRGLVLPGYKYLGPFNGLDKGEPVNEADAAALEHDKAYDRQLDSGDNPYLKYNHADAEFQERLKEDTSFGGNLGRAVFQAKKRVLEPLGLVEEPVKTAPGKKRPVEHSPVEPDSSSGTGKAGQQPARKRLNFGQTGDADSVPDPQPLGQPPAAPSGLGTNTMATGSGAPMADNNEGADGVGNSSGNWHCDSTWMGDRVITTSTRTWALPTYNNHLYKQISSQSGASNDNHYFGYSTPWGYFDFNRFHCHFSPRDWQRLINNNWGFRPKRLKFKLFNIQVKEVTQNDGTTTIANNLTSTVQVFTDSEYQLPYVLGSAHQGCLPPFPADVFMVPQYGYLTLNNGSQAVGRSSFYCLEYFPSQMLRTGNNFTFSYTFEDVPFHSSYAHSQSLDRLMNPLIDQYLYYLSRTDTPSGTTTQSRLQFSQAGASDIRNQSRNWLPGPCYRQQRVSKTSADNNNSEYSWTGATKYHLNGRDSLVNPGPAMASHKDDEEKFFPQSGVLIFGKQGSEKTSVDIEKVMITDEEEIRTTNPVATEQYGSVSTNLQRGNLAISDQTKHARQAATADVNTQGVLPGMVWQDRDVYLQGPIWAKIPHTDGHFHPSPLMGGFGLKHPPPQILIKNTPVPANPSTTFSAAKFASFITQYSTGQVSVEIEWELQKENSKRWNPEVQYTSNYNKSVNVDFTVDTNGVYSEPRPIGTRYLTRNQ

SEQ ID NO: 44 - protein, 745 aa, Artificial Sequence
  AAV capsid variant
MAADGYLPDWLEDTLSEGIRQWWKLKPGPPPPKPAERHKDDSRGLVLPGYKYLGPFNGLDKGEPVNEADAAALEHDKAYDRQLDSGDNPYLKYNHADAEFQERLKEDTSFGGNLGRAVFQAKKRVLEPLGLVEEPVKTAPGKKRPVEHSPVEPDSSSGTGKAGQQPARKRLNFGQTGDADSVPDPQPLGQPPAAPSGLGTNTMATGSGAPMADNNEGADGVGNSSGNWHCDSTWMGDRVITTSTRTWALPTYNNHLYKQISSQSGASNDNHYFGYSTPWGYFDFNRFHCHFSPRDWQRLINNNWGFRPKRLNFKLFNIQVKEVTQNDGTTTIANNLTSTVQVFTDSEYQLPYVLGSAHQGCLPPFPADVFMVPQYGYLTLNNGSQAVGRSSFYCLEYFPSQMLRTGNNFTFSYTFEDVPFHSSYAHSQSLDRLMNPLIDQYLYYLSRTNTPSGTTTQSRLQFSQAGASDIRDQSRNWLPGPCYRQQRVSKTSADNNNSEYSWTGATKYHLNGRDSLVNPGPAMASHKDDEEKFFPQSGVLIFGKQGSEKTNVDIEKVMITDEEEIRTTNPVATEQYGSVSTNLQRGNLGISDQTKHARQAATADVNTQGVLPGMVWQDRDVYLQGPIWAKIPHTDGHFHPSPLMGGFGLKHPPPQILIKNTPVPANPSTTFSAAKFASFITQYSTGQVSVEIEWELQKENSKRWNPEIQYTSNYNKSVNVDFTVDTNGVYSEPRPIGTRYLTRNL

SEQ ID NO: 45 - protein, 745 aa, Artificial Sequence
  AAV capsid variant
MAADGYLPDWLEDTLSEGIRQWWKLKPGPPPPKPAERHKDDSRGLVLPGYKYLGPFNGLDKGEPVNEADAAALEHDKAYDRQLDSGDNPYLKYNHADAEFQERLKEDTSFGGNLGRAVFQAKKRVLEPLGLVEEPVKTAPGKKRPVEHSPVEPDSSSGTGKAGQQPARKRLNFGQTGDADSVPDPQPLGQPPAAPSGLGTNTMATGSGAPMADNNEGADGVGNSSGNWHCDSTWMGDRVITTSTRTWALPTYNNHLYKQISSQSGASNDNHYFGYSTPWGYFDFNRFHCHFSPRDWQRLINNNWGFRPKRLNFKLFNIQVKEVTQNDGTTTIANNLTSTVQVFTDSEYQLPYVLGSAHQGCLPPFPADVFMVPQYGYLTLNNGSQAVGRSSFYCLEYFPSQMLRTGNNFTFSYTFEDVPFHSSYAHSQSLDRLMNPLIDQYLYYLSRTNTPSGTTTQSRLQFSQAGASDIRDQSRNWLPGPCYRQQRVSKTSADNNNSEYSWTGATKYHLNGRDSLVNPGPAMASHKDDEEKFFPQSGVLIFGKQGSEKTNVDIEKVMITDEEEIRTTNPVATEQYGSVSTNLQRGNLAQADTTKNARQAATADVNTQGVLPGMVWQDRDVYLQGPIWAKIPHTDGHFHPSPLMGGFGLKHPPPQILIKNTPVPANPSTTFSAAKFASFITQYSTGQVSVEIEWELQKENSKRWNPEVQYTSNYNKSVNVDFTVDTNGVYSEPRPIGTRYLTRNL

SEQ ID NO: 46 - protein, 745 aa, Artificial Sequence
  AAV capsid variant
MAADGYLPDWLEDTLSEGIRQWWKLKPGPPPPKPAERHKDDSRGLVLPGYKYLGPFNGLDKGEPVNEADAAALEHDKAYDRQLDSGDNPYLKYNHADAEFQERLKEDTSFGGNLGRAVFQAKKRVLEPLGLVEEPVKTAPGKKRPVEHSPVEPDSSSGTGKAGQQPARKRLNFGQTGDADSVPDPQPLGQPPAAPSGLGTNTMATGSGAPMADNNEGADGVGNSSGNWHCDSTWMGDRVITTSTRTWALPTYNNHLYKQISSQSGASNDNHYFGYSTPWGYFDFNRFHCHFSPRDWQRLINNNWGFRPKRLNFKLFNIQVKEVTQNDGTTTIANNLTSTVQVFTDSEYQLPYVLGSAHQGCLPPFPADVFMVPQYGYLTLNNGSQAVGRSSFYCLEYFPSQMLRTGNNFTFSYTFEDVPFHSSYAHSQSLDRLMNPLIDQYLYYLSRTNTPSGTTTQSRLQFSQAGASDIRDQSRNWLPGPCYRQQRVSKTSADNNNSEYSWTGATKYHLNGRDSLVNPGPAMASHKDDEEKFFPQSGVLIFGKQGSEKTNVDIEKVMITDEEEIRTTNPVATEQYGSVSTNLQRGNLAHDITKNIARQAATADVNTQGVLPGMVWQDRDVYLQGPIWAKIPHTDGHFHPSPLMGGFGLKHPPPQILIKNTPVPANPSTTFSAAKFASFITQYSTGQVSVEIEWELQKENSKRWNPEIQYTSNYNKSVNVDFTVDTNGVYSEPRPIGTRYLTRNL

SEQ ID NO: 47 - protein, 745 aa, Artificial Sequence
  AAV capsid variant
MAADGYLPDWLEDTLSEGIRQWWKLKPGPPPPKPAERHKDDSRGLVLPGYKYLGPFNGLDKGEPVNEADAAALEHDKAYDRQLDSGDNPYLKYNHADAEFQERLKEDTSFGGNLGRAVFQAKKRVLEPLGLVEEPVKTAPGKKRPVEHSPVEPDSSSGTGKAGQQPARKRLNFGQTGDADSVPDPQPLGQPPAAPSGLGTNTMATGSGAPMADNNEGADGVGNSSGNWHCDSTWMGDRVITTSTRTWALPTYNNHLYKQISSQSGASNDNHYFGYSTPWGYFDFNRFHCHFSPRDWQRLINNNWGFRPKRLNFKLFNIQVKEVTQNDGTTTIANNLTSTVQVFTDSEYQLPYVLGSAHQGCLPPFPADVFMVPQYGYLTLNNGSQAVGRSSFYCLEYFPSQMLRTGNNFTFSYTFEDVPFHSSYAHSQSLDRLMNPLIDQYLYYLSRTNTPSGTTTQSRLQFSQAGASDIRDQSRNWLPGPCYRQQRVSKTSADNNNSEYSWTGATKYHLNGRDSLVNPGPAMASHKDDEEKFFPQSGVLIFGKQGSEKTNVDIEKVMITDEEEIRTTNPVATEQYGSVSTNLQRGNLANQDYTKTARQAATADVNTQGVLPGMVWQDRDVYLQGPIWAKIPHTDGHFHPSPLMGGFGLKHPPPQILIKNTPVPANPSTTFSAAKFASFITQYSTGQVSVEIEWELQKENSKRWNPEIQYTSNYNKSVNVDFTVDTNGVYSEPRPIGTRYLTRNL

SEQ ID NO: 48 - protein, 745 aa, Artificial Sequence
  AAV capsid variant
MAADGYLPDWLEDTLSEGIRQWWKLKPGPPPPKPAERHKDDSRGLVLPGYKYLGPFNGLDKGEPVNEADAAALEHDKAYDRQLDSGDNPYLKYNHADAEFQERLKEDTSFGGNLGRAVFQAKKRVLEPLGLVEEPVKTAPGKKRPVEHSPVEPDSSSGTGKAGQQPARKRLNFGQTGDADSVPDPQPLGQPPAAPSGLGTNTMATGSGAPMADNNEGADGVGNSSGNWHCDSTWMGDRVITTSTRTWALPTYNNHLYKQISSQSGASNDNHYFGYSTPWGYFDFNRFHCHFSPRDWQRLINNNWGFRPKRLNFKLFNIQVKEVTQNDGTTTIANNLTSTVQVFTDSEYQLPYVLGSAHQGCLPPFPADVFMVPQYGYLTLNNGSQAVGRSSFYCLEYFPSQMLRTGNNFTFSYTFEDVPFHSSYAHSQSLDRLMNPLIDQYLYYLSRTNTPSGTTTQSRLQFSQAGASDIRDQSRNWLPGPCYRQQRVSKTSADNNNSEYSWTGATKYHLNGRDSLVNPGPAMASHKDDEEKFFPQSGVLIFGKQGSEKTNVDIEKVMITDEEEIRTTNPVATEQYGSVSTNLQRGNLAPNSTHGSARQAATADVNTQGVLPGMVWQDRDVYLQGPIWAKIPHTDGHFHPSPLMGGFGLKHPPPQILIKNTPVPANPSTTFSAAKFASFITQYSTGQVSVEIEWELQKENSKRWNPEIQYTSNYNKSVNVDFTVDTNGVYSEPRPIGTRYLTRNL

SEQ ID NO: 49 - protein, 745 aa, Artificial Sequence
  AAV capsid variant
MAADGYLPDWLEDTLSEGIRQWWKLKPGPPPPKPAERHKDDSRGLVLPGYKYLGPFNGLDKGEPVNEADAAALEHDKAYDRQLDSGDNPYLKYNHADAEFQERLKEDTSFGGNLGRAVFQAKKRVLEPLGLVEEPVKTAPGKKRPVEHSPVEPDSSSGTGKAGQQPARKRLNFGQTGDADSVPDPQPLGQPPAAPSGLGTNTMATGSGAPMADNNEGADGVGNSSGNWHCDSTWMGDRVITTSTRTWALPTYNNHLYKQISSQSGASNDNHYFGYSTPWGYFDFNRFHCHFSPRDWQRLINNNWGFRPKRLNFKLFNIQVKEVTQNDGTTTIANNLTSTVQVFTDSEYQLPYVLGSAHQGCLPPFPADVFMVPQYGYLTLNNGSQAVGRSSFYCLEYFPSQMLRTGNNFTFSYTFEDVPFHSSYAHSQSLDRLMNPLIDQYLYYLSRTNTPSGTTTQSRLQFSQAGASDIRDQSRNWLPGPCYRQQRVSKTSADNNNSEYSWTGATKYHLNGRDSLVNPGPAMASHKDDEEKFFPQSGVLIFGKQGSEKTNVDIEKVMITDEEEIRTTNPVATEQYGSVSTNLQRGNLANKTTNKDARQAATADVNTQGVLPGMVWQDRDVYLQGPIWAKIPHTDGHFHPSPLMGGFGLKHPPPQILIKNTPVPANPSTTFSAAKFASFITQYSTGQVSVEIEWELQKENSKRWNPEIQYTSNYNKSVNVDFTVDTNGVYSEPRPIGTRYLTRNL

SEQ ID NO: 50 - protein, 745 aa, Artificial Sequence
  AAV capsid variant
MAADGYLPDWLEDTLSEGIRQWWKLKPGPPPPKPAERHKDDSRGLVLPGYKYLGPFNGLDKGEPVNEADAAALEHDKAYDRQLDSGDNPYLKYNHADAEFQERLKEDTSFGGNLGRAVFQAKKRVLEPLGLVEEPVKTAPGKKRPVEHSPVEPDSSSGTGKAGQQPARKRLNFGQTGDADSVPDPQPLGQPPAAPSGLGTNTMATGSGAPMADNNEGADGVGNSSGNWHCDSTWMGDRVITTSTRTWALPTYNNHLYKQISSQSGASNDNHYFGYSTPWGYFDFNRFHCHFSPRDWQRLINNNWGFRPKRLNFKLFNIQVKEVTQNDGTTTIANNLTSTVQVFTDSEYQLPYVLGSAHQGCLPPFPADVFMVPQYGYLTLNNGSQAVGRSSFYCLEYFPSQMLRTGNNFTFSYTFEDVPFHSSYAHSQSLDRLMNPLIDQYLYYLSRTNTPSGTTTQSRLQFSQAGASDIRDQSRNWLPGPCYRQQRVSKTSADNNNSEYSWTGATKYHLNGRDSLVNPGPAMASHKDDEEKFFPQSGVLIFGKQGSEKTNVDIEKVMITDEEEIRTTNPVATEQYGSVSTNLQRGNLATNRTSPDARQAATADVNTQGVLPGMVWQDRDVYLQGPIWAKIPHTDGHFHPSPLMGGFGLKHPPPQILIKNTPVPANPSTTFSAAKFASFITQYSTGQVSVEIEWELQKENSKRWNPEIQYTSNYNKSVNVDFTVDTNGVYSEPRPIGTRYLTRNL

SEQ ID NO: 51 - protein, 745 aa, Artificial Sequence
  AAV capsid variant
MAADGYLPDWLEDTLSEGIRQWWKLKPGPPPPKPAERHKDDSRGLVLPGYKYLGPFNGLDKGEPVNEADAAALEHDKAYDRQLDSGDNPYLKYNHADAEFQERLKEDTSFGGNLGRAVFQAKKRVLEPLGLVEEPVKTAPGKKRPVEHSPVEPDSSSGTGKAGQQPARKRLNFGQTGDADSVPDPQPLGQPPAAPSGLGTNTMATGSGAPMADNNEGADGVGNSSGNWHCDSTWMGDRVITTSTRTWALPTYNNHLYKQISSQSGASNDNHYFGYSTPWGYFDFNRFHCHFSPRDWQRLINNNWGFRPKRLNFKLFNIQVKEVTQNDGTTTIANNLTSTVQVFTDSEYQLPYVLGSAHQGCLPPFPADVFMVPQYGYLTLNNGSQAVGRSSFYCLEYFPSQMLRTGNNFTFSYTFEDVPFHSSYAHSQSLDRLMNPLIDQYLYYLSRTNTPSGTTTQSRLQFSQAGASDIRDQSRNWLPGPCYRQQRVSKTSADNNNSEYSWTGATKYHLNGRDSLVNPGPAMASHKDDEEKFFPQSGVLIFGKQGSEKTNVDIEKVMITDEEEIRTTNPVATEQYGSVSTNLQRGNLAGKSKVIDARQAATADVNTQGVLPGMVWQDRDVYLQGPIWAKIPHTDGHFHPSPLMGGFGLKHPPPQILIKNTPVPANPSTTFSAAKFASFITQYSTGQVSVEIEWELQKENSKRWNPEIQYTSNYNKSVNVDFTVDTNGVYSEPRPIGTRYLTRNL

SEQ ID NO: 52 - protein, 745 aa, Artificial Sequence
  AAV capsid variant
MAADGYLPDWLEDTLSEGIRQWWKLKPGPPPPKPAERHKDDSRGLVLPGYKYLGPFNGLDKGEPVNEADAAALEHDKAYDRQLDSGDNPYLKYNHADAEFQERLKEDTSFGGNLGRAVFQAKKRVLEPLGLVEEPVKTAPGKKRPVEHSPVEPDSSSGTGKAGQQPARKRLNFGQTGDADSVPDPQPLGQPPAAPSGLGTNTMATGSGAPMADNNEGADGVGNSSGNWHCDSTWMGDRVITTSTRTWALPTYNNHLYKQISSQSGASNDNHYFGYSTPWGYFDFNRFHCHFSPRDWQRLINNNWGFRPKRLNFKLFNIQVKEVTQNDGTTTIANNLTSTVQVFTDSEYQLPYVLGSAHQGCLPPFPADVFMVPQYGYLTLNNGSQAVGRSSFYCLEYFPSQMLRTGNNFTFSYTFEDVPFHSSYAHSQSLDRLMNPLIDQYLYYLSRTNTPSGTTTQSRLQFSQAGASDIRDQSRNWLPGPCYRQQRVSKTSADNNNSEYSWTGATKYHLNGRDSLVNPGPAMASHKDDEEKFFPQSGVLIFGKQGSEKTNVDIEKVMITDEEEIRTTNPVATEQYGSVSTNLQRGNLAASDSTKAARQAATADVNTQGVLPGMVWQDRDVYLQGPIWAKIPHTDGHFHPSPLMGGFGLKHPPPQILIKNTPVPANPSTTFSAAKFASFITQYSTGQVSVEIEWELQKENSKRWNPEIQYTSNYNKSVNVDFTVDTNGVYSEPRPIGTRYLTRNL

SEQ ID NO: 53 - protein, 745 aa, Artificial Sequence
  AAV capsid variant
MAADGYLPDWLEDTLSEGIRQWWKLKPGPPPPKPAERHKDDSRGLVLPGYKYLGPFNGLDKGEPVNEADAAALEHDKAYDRQLDSGDNPYLKYNHADAEFQERLKEDTSFGGNLGRAVFQAKKRVLEPLGLVEEPVKTAPGKKRPVEHSPVEPDSSSGTGKAGQQPARKRLNFGQTGDADSVPDPQPLGQPPAAPSGLGTNTMATGSGAPMADNNEGADGVGNSSGNWHCDSTWMGDRVITTSTRTWALPTYNNHLYKQISSQSGASNDNHYFGYSTPWGYFDFNRFHCHFSPRDWQRLINNNWGFRPKRLNFKLFNIQVKEVTQNDGTTTIANNLTSTVQVFTDSEYQLPYVLGSAHQGCLPPFPADVFMVPQYGYLTLNNGSQAVGRSSFYCLEYFPSQMLRTGNNFTFSYTFEDVPFHSSYAHSQSLDRLMNPLIDQYLYYLSRTNTPSGTTTQSRLQFSQAGASDIRDQSRNWLPGPCYRQQRVSKTSADNNNSEYSWTGATKYHLNGRDSLVNPGPAMASHKDDEEKFFPQSGVLIFGKQGSEKTNVDIEKVMITDEEEIRTTNPVATEQYGSVSTNLQRGNLAKDRAPSTARQAATADVNTQGVLPGMVWQDRDVYLQGPIWAKIPHTDGHFHPSPLMGGFGLKHPPPQILIKNTPVPANPSTTFSAAKFASFITQYSTGQVSVEIEWELQKENSKRWNPEIQYTSNYNKSVNVDFTVDTNGVYSEPRPIGTRYLTRNL

SEQ ID NO: 54 - protein, 745 aa, Artificial Sequence
  AAV capsid variant
MAADGYLPDWLEDTLSEGIRQWWKLKPGPPPPKPAERHKDDSRGLVLPGYKYLGPFNGLDKGEPVNEADAAALEHDKAYDRQLDSGDNPYLKYNHADAEFQERLKEDTSFGGNLGRAVFQAKKRVLEPLGLVEEPVKTAPGKKRPVEHSPVEPDSSSGTGKAGQQPARKRLNFGQTGDADSVPDPQPLGQPPAAPSGLGTNTMATGSGAPMADNNEGADGVGNSSGNWHCDSTWMGDRVITTSTRTWALPTYNNHLYKQISSQSGASNDNHYFGYSTPWGYFDFNRFHCHFSPRDWQRLINNNWGFRPKRLNFKLFNIQVKEVTQNDGTTTIANNLTSTVQVFTDSEYQLPYVLGSAHQGCLPPFPADVFMVPQYGYLTLNNGSQAVGRSSFYCLEYFPSQMLRTGNNFTFSYTFEDVPFHSSYAHSQSLDRLMNPLIDQYLYYLSRTNTPSGTTTQSRLQFSQAGASDIRDQSRNWLPGPCYRQQRVSKTSADNNNSEYSWTGATKYHLNGRDSLVNPGPAMASHKDDEEKFFPQSGVLIFGKQGSEKTNVDIEKVMITDEEEIRTTNPVATEQYGSVSTNLQRGNLAHQDTTKNARQAATADVNTQGVLPGMVWQDRDVYLQGPIWAKIPHTDGHFHPSPLMGGFGLKHPPPQILIKNTPVPANPSTTFSAAKFASFITQYSTGQVSVEIEWELQKENSKRWNPEIQYTSNYNKSVNVDFTVDTNGVYSEPRPIGTRYLTRNL

SEQ ID NO: 55 - protein, 745 aa, Artificial Sequence
  AAV capsid variant
MAADGYLPDWLEDTLSEGIRQWWKLKPGPPPPKPAERHKDDSRGLVLPGYKYLGPFNGLDKGEPVNEADAAALEHDKAYDRQLDSGDNPYLKYNHADAEFQERLKEDTSFGGNLGRAVFQAKKRVLEPLGLVEEPVKTAPGKKRPVEHSPVEPDSSSGTGKAGQQPARKRLNFGQTGDADSVPDPQPLGQPPAAPSGLGTNTMATGSGAPMADNNEGADGVGNSSGNWHCDSTWMGDRVITTSTRTWALPTYNNHLYKQISSQSGASNDNHYFGYSTPWGYFDFNRFHCHFSPRDWQRLINNNWGFRPKRLNFKLFNIQVKEVTQNDGTTTIANNLTSTVQVFTDSEYQLPYVLGSAHQGCLPPFPADVFMVPQYGYLTLNNGSQAVGRSSFYCLEYFPSQMLRTGNNFTFSYTFEDVPFHSSYAHSQSLDRLMNPLIDQYLYYLSRTNTPSGTTTQSRLQFSQAGASDIRDQSRNWLPGPCYRQQRVSKTSADNNNSEYSWTGATKYHLNGRDSLVNPGPAMASHKDDEEKFFPQSGVLIFGKQGSEKTNVDIEKVMITDEEEIRTTNPVATEQYGSVSTNLQRGNLPISNENEHARQAATADVNTQGVLPGMVWQDRDVYLQGPIWAKIPHTDGHFHPSPLMGGFGLKHPPPQILIKNTPVPANPSTTFSAAKFASFITQYSTGQVSVEIEWELQKENSKRWNPEIQYTSNYNKSVNVDFTVDTNGVYSEPRPIGTRYLTRNL

SEQ ID NO: 56 - protein, 745 aa, Artificial Sequence
  AAV capsid variant
MAADGYLPDWLEDTLSEGIRQWWKLKPGPPPPKPAERHKDDSRGLVLPGYKYLGPFNGLDKGEPVNEADAAALEHDKAYDRQLDSGDNPYLKYNHADAEFQERLKEDTSFGGNLGRAVFQAKKRVLEPLGLVEEPVKTAPGKKRPVEHSPVEPDSSSGTGKAGQQPARKRLNFGQTGDADSVPDPQPLGQPPAAPSGLGTNTMATGSGAPMADNNEGADGVGNSSGNWHCDSTWMGDRVITTSTRTWALPTYNNHLYKQISSQSGASNDNHYFGYSTPWGYFDFNRFHCHFSPRDWQRLINNNWGFRPKRLNFKLFNIQVKEVTQNDGTTTIANNLTSTVQVFTDSEYQLPYVLGSAHQGCLPPFPADVFMVPQYGYLTLNNGSQAVGRSSFYCLEYFPSQMLRTGNNFTFSYTFEDVPFHSSYAHSQSLDRLMNPLIDQYLYYLSRTNTPSGTTTQSRLQFSQAGASDIRDQSRNWLPGPCYRQQRVSKTSADNNNSEYSWTGATKYHLNGRDSLVNPGPAMASHKDDEEKFFPQSGVLIFGKQGSEKTNVDIEKVMITDEEEIRTTNPVATEQYGSVSTNLQRGNLPQANANENARQAATADVNTQGVLPGMVWQDRDVYLQGPIWAKIPHTDGHFHPSPLMGGFGLKHPPPQILIKNTPVPANPSTTFSAAKFASFITQYSTGQVSVEIEWELQKENSKRWNPEIQYTSNYNKSVNVDFTVDTNGVYSEPRPIGTRYLTRNL

SEQ ID NO: 57 - protein, 745 aa, Artificial Sequence
  AAV capsid variant
MAADGYLPDWLEDTLSEGIRQWWKLKPGPPPPKPAERHKDDSRGLVLPGYKYLGPFNGLDKGEPVNEADAAALEHDKAYDRQLDSGDNPYLKYNHADAEFQERLKEDTSFGGNLGRAVFQAKKRVLEPLGLVEEPVKTAPGKKRPVEHSPVEPDSSSGTGKAGQQPARKRLNFGQTGDADSVPDPQPLGQPPAAPSGLGTNTMATGSGAPMADNNEGADGVGNSSGNWHCDSTWMGDRVITTSTRTWALPTYNNHLYKQISSQSGASNDNHYFGYSTPWGYFDFNRFHCHFSPRDWQRLINNNWGFRPKRLNFKLFNIQVKEVTQNDGTTTIANNLTSTVQVFTDSEYQLPYVLGSAHQGCLPPFPADVFMVPQYGYLTLNNGSQAVGRSSFYCLEYFPSQMLRTGNNFTFSYTFEDVPFHSSYAHSQSLDRLMNPLIDQYLYYLSRTNTPSGTTTQSRLQFSQAGASDIRDQSRNWLPGPCYRQQRVSKTSADNNNSEYSWTGATKYHLNGRDSLVNPGPAMASHKDDEEKFFPQSGVLIFGKQGSEKTNVDIEKVMITDEEEIRTTNPVATEQYGSVSTNLQRGNLAHPDTTKNARQAATADVNTQGVLPGMVWQDRDVYLQGPIWAKIPHTDGHFHPSPLMGGFGLKHPPPQILIKNTPVPANPSTTFSAAKFASFITQYSTGQVSVEIEWELQKENSKRWNPEIQYTSNYNKSVNVDFTVDTNGVYSEPRPIGTRYLTRNL

SEQ ID NO: 58 - protein, 737 aa, Artificial Sequence
  Ancestral capsid protein
  misc_feature (264)..(264): Xaa can be any naturally occurring amino acid
  misc_feature (266)..(266): Xaa can be any naturally occurring amino acid
  misc_feature (268)..(268): Xaa can be any naturally occurring amino acid
  misc_feature (448)..(448): Xaa can be any naturally occurring amino acid
  misc_feature (459)..(460): Xaa can be any naturally occurring amino acid
  misc_feature (467)..(467): Xaa can be any naturally occurring amino acid
  misc_feature (470)..(471): Xaa can be any naturally occurring amino acid
  misc_feature (474)..(474): Xaa can be any naturally occurring amino acid
  misc_feature (495)..(495): Xaa can be any naturally occurring amino acid
  misc_feature (516)..(516): Xaa can be any naturally occurring amino acid
  misc_feature (533)..(533): Xaa can be any naturally occurring amino acid
  misc_feature (547)..(547): Xaa can be any naturally occurring amino acid
  misc_feature (551)..(551): Xaa can be any naturally occurring amino acid
  misc_feature (555)..(555): Xaa can be any naturally occurring amino acid
  misc_feature (557)..(557): Xaa can be any naturally occurring amino acid
  misc_feature (561)..(561): Xaa can be any naturally occurring amino acid
  misc_feature (563)..(563): Xaa can be any naturally occurring amino acid
  misc_feature (577)..(577): Xaa can be any naturally occurring amino acid
  misc_feature (583)..(583): Xaa can be any naturally occurring amino acid
  misc_feature (593)..(593): Xaa can be any naturally occurring amino acid
  misc_feature (596)..(596): Xaa can be any naturally occurring amino acid
  misc_feature (661)..(662): Xaa can be any naturally occurring amino acid
  misc_feature (664)..(665): Xaa can be any naturally occurring amino acid
  misc_feature (710)..(710): Xaa can be any naturally occurring amino acid
  misc_feature (717)..(719): Xaa can be any naturally occurring amino acid
  misc_feature (723)..(723): Xaa can be any naturally occurring amino acid
MAADGYLPDWLEDNLSEGIREWWDLKPGAPKPKANQQKQDDGRGLVLPGYKYLGPFNGLDKGEPVNAADAAALEHDKAYDQQLKAGDNPYLRYNHADAEFQERLQEDTSFGGNLGRAVFQAKKRVLEPLGLVEEGAKTAPGKKRPVEPSPQRSPDSSTGIGKKGQQPAKKRLNFGQTGDSESVPDPQPLGEPPAGPSGLGSGTMAAGGGAPMADNNEGADGVGNASGNWHCDSTWLGDRVITTSTRTWALPTYNNHLYKQISSXSXGXTNDNHYFGYSTPWGYFDFNRFHCHFSPRDWQRLINNNWGFRPKRLNFKLFNIQVKEVTTNDGVTTIANNLTSTVQVFSDSEYQLPYVLGSAHQGCLPPFPADVFMIPQYGYLTLNNGSQAVGRSSFYCLEYFPSQMLRTGNNFTFSYTFEDVPFHSSYAHSQSLDRLMNPLIDQYLYYLXRTQSTGGTAGXXELLFSQXGPXXMSXQAKNWLPGPCYRQQRVSKTLXQNNNSNFAWTGATKYHLNGRXSLVNPGVAMATHKDDEXRFFPSSGVLIFGKXGAGXNNTXLXNVMXTXEEEIKTTNPVATEXYGVVAXNLQSSNTAPXTGXVNSQGALPGMVWQNRDVYLQGPIWAKIPHTDGNFHPSPLMGGFGLKHPPPQILIKNTPVPANPPXXFXXAKFASFITQYSTGQVSVEIEWELQKENSKRWNPEIQYTSNYAKSXNVDFAVXXXGVYXEPRPIGTRYLTRNL

SEQ ID NO: 59 - protein, 737 aa, Artificial Sequence
  Ancestral variant capsid
MAADGYLPDWLEDNLSEGIREWWDLKPGAPKPKANQQKQDDGRGLVLPGYKYLGPFNGLDKGEPVNAADAAALEHDKAYDQQLKAGDNPYLRYNHADAEFQERLQEDTSFGGNLGRAVFQAKKRVLEPLGLVEEGAKTAPGKKRPVEPSPQRSPDSSTGIGKKGQQPAKKRLNFGQTGDSESVPDPQPLGEPPAGPSGLGSGTMAAGGGAPMADNNEGADGVGNASGNWHCDSTWLGDRVITTSTRTWALPTYNNHLYKQISSASAGSTNDNHYFGYSTPWGYFDFNRFHCHFSPRDWQRLINNNWGFRPKRLNFKLFNIQVKEVTTNDGVTTIANNLTSTVQVFSDSEYQLPYVLGSAHQGCLPPFPADVFMIPQYGYLTLNNGSQAVGRSSFYCLEYFPSQMLRTGNNFTFSYTFEDVPFHSSYAHSQSLDRLMNPLIDQYLYYLARTQSTGGTAGTRELLFSQAGPSNMSAQAKNWLPGPCYRQQRVSKTLSQNNNSNFAWTGATKYHLNGRDSLVNPGVAMATHKDDEDRFFPSSGVLIFGKQGAGANNTALENVMMTSEEEIKTTNPVATEQYGVVASNLQSSNTAPVTGTVNSQGALPGMVWQNRDVYLQGPIWAKIPHTDGNFHPSPLMGGFGLKHPPPQILIKNTPVPANPPAVFTPAKFASFITQYSTGQVSVEIEWELQKENSKRWNPEIQYTSNYAKSTNVDFAVDNEGVYSEPRPIGTRYLTRNL

SEQ ID NO: 60 - protein, 10 aa, Artificial Sequence
  Heterologous peptide insertion
IAHDITKNIA

SEQ ID NO: 61 - protein, 7 aa, Artificial Sequence
  Heterologous peptide insertion
DITKNIA

SEQ ID NO: 62 - protein, 8 aa, Artificial Sequence
  Heterologous peptide insertion
NKTTNKDA

SEQ ID NO: 63 - protein, 8 aa, Artificial Sequence
  Heterologous peptide insertion
PQANANEN

SEQ ID NO: 64 - protein, 8 aa, Artificial Sequence
  Heterologous peptide insertion
PISNENEH

SEQ ID NO: 65 - DNA, 1377 bp, Artificial Sequence
  codon-optimized sequence encoding Aflibercept
atggtttcttactgggacaccggcgtgctgctgtgtgccctgctttcttgtctgctgctgaccggctctagcagcggctctgataccggcagacccttcgtggaaatgtacagcgagatccccgagatcatccacatgaccgagggcagagagctggtcatcccttgcagagtgacaagccccaacatcaccgtgactctgaagaagttccctctggacacactgatccccgacggcaagagaatcatctgggacagccggaagggcttcatcatcagcaacgccacctacaaagagatcggcctgctgacctgtgaagccaccgtgaatggccacctgtacaagaccaactacctgacacacagacagaccaacaccatcatcgacgtggtgctgagccctagccacggcattgaactgtctgtgggcgagaagctggtgctgaactgtaccgccagaaccgagctgaacgtgggcatcgacttcaactgggagtaccccagcagcaagcaccagcacaagaaactggtcaaccgggacctgaaaacccagagcggcagcgagatgaagaaattcctgagcaccctgaccatcgacggcgtgaccagaagtgaccagggcctgtacacatgtgccgccagctctggcctgatgaccaagaaaaacagcaccttcgtgcgggtgcacgagaaggacaagacccacacctgtcctccatgtcctgctccagaactgctcggcggaccttccgtgttcctgtttcctccaaagcctaaggacaccctgatgatcagcagaacccctgaagtgacctgcgtggtggtggatgtgtcccacgaggatcccgaagtgaagttcaattggtacgtggacggcgtggaagtgcacaacgccaagaccaagcctagagaggaacagtacaatagcacctacagagtggtgtccgtgctgaccgtgctgcaccaggattggctgaacggcaaagagtacaagtgcaaggtgtccaacaaggccctgcctgctcctatcgagaaaaccatctccaaggccaagggccagcctagggaaccccaggtttacacactgcctccaagcagggacgagctgacaaagaaccaggtgtccctgacctgcctggtcaagggcttctacccttccgatatcgccgtggaatgggagagcaatggccagcctgagaacaactacaagacaacccctcctgtgctggacagcgacggctcattcttcctgtacagcaagctgacagtggacaagagcagatggcagcagggcaacgtgttcagctgctccgtgatgcacgaggccctgcacaaccactacacccagaagtccctgagcctgtctcctggcaaatga

SEQ ID NO: 66 - protein, 458 aa, Artificial Sequence
  Aflibercept
MVSYWDTGVLLCALLSCLLLTGSSSGSDTGRPFVEMYSEIPEIIHMTEGRELVIPCRVTSPNITVTLKKFPLDTLIPDGKRIIWDSRKGFIISNATYKEIGLLTCEATVNGHLYKTNYLTHRQTNTIIDVVLSPSHGIELSVGEKLVLNCTARTELNVGIDFNWEYPSSKHQHKKLVNRDLKTQSGSEMKKFLSTLTIDGVTRSDQGLYTCAASSGLMTKKNSTFVRVHEKDKTHTCPPCPAPELLGGPSVFLFPPKPKDTLMISRTPEVTCVVVDVSHEDPEVKFNWYVDGVEVHNAKTKPREEQYNSTYRVVSVLTVLHQDWLNGKEYKCKVSNKALPAPIEKTISKAKGQPREPQVYTLPPSRDELTKNQVSLTCLVKGFYPSDIAVEWESNGQPENNYKTTPPVLDSDGSFFLYSKLTVDKSRWQQGNVFSCSVMHEALHNHYTQKSLSLSPGK

SEQ ID NO: 67 - DNA, 1575 bp, Artificial Sequence
  codon optimized sequence encoding single chain Heavy-Light Ranibizumab
atggactggacctggtccatcctgtttctggtggctgccgccacaggcacatactctgaagtgcagctggtggaatctggcggcggacttgttcaacctggcggctctctgagactgagctgtgccgcctctggctacgactttacccactacggcatgaactgggtccgacaggcccctggcaaaggccttgaatgggtcggatggatcaacacctacaccggcgagccaacatacgccgccgacttcaagcggagattcaccttcagcctggacaccagcaagagcaccgcctacctccagatgaacagcctgagagccgaggacaccgccgtgtactactgcgccaagtatccctactactacggcaccagccactggtacttcgacgtgtggggacagggcacactggtcacagtgtctagcgcctctacaaagggccccagcgttttcccactggctcctagcagcaagtctacctccggtggaacagccgctctgggctgtctggtcaaggactactttcccgagcctgtgaccgtgtcctggaatagcggagcactgacaagcggcgtgcacacctttccagccgtgctgcaaagcagcggcctgtactctctgagcagcgtcgtgacagtgccaagcagctctctgggcacccagacctacatctgcaatgtgaaccacaagcctagcaacaccaaggtggacaagaaggtggaacccaagagctgcgacaagacacacctcggcggaagctctggaagcggctctggatctaccggcacaagctctagcggaacaggcacaagcgctggcacaaccggaacaagcgcttctacatctggctctggttctggcggaggcggaggatcaggtggtggtggatctgctggcggaacagctacagctggcgcctcttctggcagcgacattcagctgacacagagcccttctagcctgagcgcctctgtgggcgacagagtgaccatcacatgtagcgccagccaggacatctccaactacctgaactggtatcagcagaagcccggcaaggcccctaaggtgctgatctactttaccagcagcctgcactccggcgtgcccagcagattttctggatctggctccggcaccgacttcaccctgacaatatctagcctccagcctgaggacttcgccacctactactgccagcagtacagcaccgtgccttggacatttggccagggcacaaaggtggaaatcaagcggacagtggccgctcctagcgtgttcatctttccacctagcgacgagcagctgaagtctggcacagcctctgtcgtgtgcctgctgaacaacttctaccccagagaagccaaggtgcagtggaaagtggacaacgccctccagtccggcaacagccaagagtctgtgaccgagcaggacagcaaggactccacctacagcctgtccagcacactgacactgagcaaggccgactacgagaagcacaaagtgtacgcctgcgaagtgacccaccagggcctttctagccctgtgaccaagagcttcaaccggggcgagtgttga

SEQ ID NO: 68 - protein, 524 aa, Artificial Sequence
  single chain Heavy-Light Ranibizumab
MDWTWSILFLVAAATGTYSEVQLVESGGGLVQPGGSLRLSCAASGYDFTHYGMNWVRQAPGKGLEWVGWINTYTGEPTYAADFKRRFTFSLDTSKSTAYLQMNSLRAEDTAVYYCAKYPYYYGTSHWYFDVWGQGTLVTVSSASTKGPSVFPLAPSSKSTSGGTAALGCLVKDYFPEPVTVSWNSGALTSGVHTFPAVLQSSGLYSLSSVVTVPSSSLGTQTYICNVNHKPSNTKVDKKVEPKSCDKTHLGGSSGSGSGSTGTSSSGTGTSAGTTGTSASTSGSGSGGGGGSGGGGSAGGTATAGASSGSDIQLTQSPSSLSASVGDRVTITCSASQDISNYLNWYQQKPGKAPKVLIYFTSSLHSGVPSRFSGSGSGTDFTLTISSLQPEDFATYYCQQYSTVPWTFGQGTKVEIKRTVAAPSVFIFPPSDEQLKSGTASVVCLLNNFYPREAKVQWKVDNALQSGNSQESVTEQDSKDSTYSLSSTLTLSKADYEKHKVYACEVTHQGLSSPVTKSFNRGEC

SEQ ID NO: 69 - DNA, 1578 bp, Artificial Sequence
  codon optimized sequence encoding single chain Light-Heavy Ranibizumab
atggtcctccagacacaggtgttcatcagcctgctgctgtggatctctggcgcctacggcgatatccagctgacacagagccctagcagcctgtctgcctctgtgggcgacagagtgaccatcacatgtagcgccagccaggacatcagcaactacctgaactggtatcagcagaagcccggcaaggcccctaaggtgctgatctactttaccagcagcctgcacagcggcgtgcccagcagattttctggctctggcagcggcaccgacttcaccctgacaatatctagcctccagcctgaggacttcgccacctactactgccagcagtacagcaccgtgccttggacatttggccagggcaccaaggtggaaatcaagcggacagtggccgctcctagcgtgttcatctttccacctagcgacgagcagctgaagtctggcacagcctctgtcgtgtgcctgctgaacaacttctaccccagagaagccaaggtgcagtggaaggtggacaacgccctccagagcggcaatagccaagagagcgtgaccgagcaggacagcaaggactctacctactctctgagcagcacactgaccctgagcaaggccgactacgagaagcacaaagtgtacgcctgcgaagtgacccaccagggcctttctagccctgtgaccaagagcttcaacagaggcgagtgtggcggcagctctggaagcggatctggaagcacaggcacaagctctagcggaaccggaacaagcgctggcacaacaggcacatctgccagcacaagcggttctggttctggcggaggcggaggatctggtggtggcggatctgctggcggaacagctacagctggtgcctcttctggatccgaggtgcagctggttgaatctggcggtggactggttcagccaggcggatctctgagactgtcttgtgccgccagcggctacgatttcacccactacggcatgaactgggtccgacaggcccctggcaaaggccttgaatgggtcggatggatcaacacctacaccggcgagccaacatacgccgccgacttcaagcggagattcaccttcagcctggacacctccaagagcaccgcctacctccagatgaacagcctgagagccgaggacaccgccgtgtactactgcgccaagtatccctactactacggcaccagccactggtacttcgacgtgtggggacagggcacactggtcacagtgtctagcgcctctacaaagggccccagcgttttcccactggctcctagcagcaagagcacatcaggcggaactgctgccctgggctgtctggtcaaggactactttcctgagcctgtgaccgtgtcctggaacagcggagcactgacatctggcgtgcacacctttccagccgtgctccaaagcagcggcctgtattctctgtccagcgtcgtgacagtgcctagcagctctctgggcacccagacctacatctgcaatgtgaaccacaagcctagcaacaccaaggtcgacaagaaggtggaacccaagagctgcgacaagacccacctctga

SEQ ID NO: 70 - DNA, 1578 bp, Artificial Sequence
  codon optimized single chain Light-Heavy Ranibizumab
atggtgctccagacccaggtgtttatttcactgctgctgtggattagcggggcttacggagacattcagctgacccagagtccttcatctctgagcgcctccgtgggcgacagggtgaccatcacatgctctgccagccaggatatctccaactatctgaattggtaccagcagaagcccggcaaggcccctaaggtgctgatctatttcaccagctccctgcacagcggagtgccatcccgcttctccggctctggcagcggcaccgactttaccctgacaatctctagcctccagccagaggatttcgccacatactattgccagcagtacagcaccgtgccctggacatttggccagggcaccaaggtggagatcaagcggacagtggccgccccaagcgtgttcatctttccccctagcgacgagcagctgaagtctggcaccgccagcgtggtgtgcctgctgaacaatttctatcccagagaggccaaggtgcagtggaaggtggataacgccctccagtccggcaattctcaggagagcgtgaccgagcaggactccaaggattctacatacagcctgtcctctaccctgacactgtccaaggccgactatgagaagcacaaggtgtacgcatgcgaggtgacccaccagggcctgagctccccagtgacaaagagctttaacaggggagagtgtggaggatctagcggatccggatctggaagcaccggcacatcctctagcggaaccggcacaagcgccggcaccacaggcacctccgcctctacaagcggcagcggatctggcggaggaggaggatccggaggaggaggatctgccggcggcaccgccacagccggcgcctcctctggctccgaggtgcagctggtggagtctggaggaggcctggtgcagcctggaggctccctgaggctgtcttgcgcagcaagcggctatgatttcacccactacggaatgaactgggtgcgccaggcacctggcaagggcctggagtgggtgggctggatcaatacctatacaggcgagccaacctacgccgccgactttaagcggagattcacattttccctggataccagcaagtccacagcctacctccagatgaacagcctgagggcagaggacaccgccgtgtactattgcgccaagtatccttactattacggcacaagccactggtacttcgacgtgtggggacagggcaccctggtgacagtgagctccgccagcaccaagggcccatccgtgtttcctctggccccatctagcaagtctaccagcggaggaacagccgccctgggatgtctggtgaaggactacttcccagagcccgtgaccgtgtcctggaattctggcgccctgacctccggcgtgcacacatttcccgccgtgctccagtcctctggcctgtatagcctgagctccgtggtgaccgtgccttctagctccctgggcacccagacatacatctgtaacgtgaatcacaagccttcaaataccaaagtcgataaaaaagtggaaccaaaatcctgtgataaaacccatctgtga

SEQ ID NO: 71 - protein, 525 aa, Artificial Sequence
  single chain Light-Heavy Ranibizumab
MVLQTQVFISLLLWISGAYGDIQLTQSPSSLSASVGDRVTITCSASQDISNYLNWYQQKPGKAPKVLIYFTSSLHSGVPSRFSGSGSGTDFTLTISSLQPEDFATYYCQQYSTVPWTFGQGTKVEIKRTVAAPSVFIFPPSDEQLKSGTASVVCLLNNFYPREAKVQWKVDNALQSGNSQESVTEQDSKDSTYSLSSTLTLSKADYEKHKVYACEVTHQGLSSPVTKSFNRGECGGSSGSGSGSTGTSSSGTGTSAGTTGTSASTSGSGSGGGGGSGGGGSAGGTATAGASSGSEVQLVESGGGLVQPGGSLRLSCAASGYDFTHYGMNWVRQAPGKGLEWVGWINTYTGEPTYAADFKRRFTFSLDTSKSTAYLQMNSLRAEDTAVYYCAKYPYYYGTSHWYFDVWGQGTLVTVSSASTKGPSVFPLAPSSKSTSGGTAALGCLVKDYFPEPVTVSWNSGALTSGVHTFPAVLQSSGLYSLSSVVTVPSSSLGTQTYICNVNHKPSNTKVDKKVEPKSCDKTHL

SEQ ID NO: 72 - DNA, 2277 bp, Artificial Sequence
  sequence encoding single chain Light-Heavy Ranibizumab-Fc
atggtcctccagacacaggtgttcatcagcctgctgctgtggatctctggcgcctacggcgatatccagctgacacagagccctagcagcctgtctgcctctgtgggcgacagagtgaccatcacatgtagcgccagccaggacatcagcaactacctgaactggtatcagcagaagcccggcaaggcccctaaggtgctgatctactttaccagcagcctgcacagcggcgtgcccagcagattttctggctctggcagcggcaccgacttcaccctgacaatatctagcctccagcctgaggacttcgccacctactactgccagcagtacagcaccgtgccttggacatttggccagggcaccaaggtggaaatcaagcggacagtggccgctcctagcgtgttcatctttccacctagcgacgagcagctgaagtctggcacagcctctgtcgtgtgcctgctgaacaacttctaccccagagaagccaaggtgcagtggaaggtggacaacgccctccagagcggcaatagccaagagagcgtgaccgagcaggacagcaaggactctacctactctctgagcagcacactgaccctgagcaaggccgactacgagaagcacaaagtgtacgcctgcgaagtgacccaccagggcctttctagccctgtgaccaagagcttcaacagaggcgagtgtggcggcagctctggaagcggatctggaagcacaggcacaagctctagcggaaccggaacaagcgctggcacaacaggcacatctgccagcacaagcggttctggttctggcggaggcggaggatctggtggtggcggatctgctggcggaacagctacagctggtgcctcttctggatccgaggtgcagctggttgaatctggcggtggactggttcagccaggcggatctctgagactgtcttgtgccgccagcggctacgatttcacccactacggcatgaactgggtccgacaggcccctggcaaaggccttgaatgggtcggatggatcaacacctacaccggcgagccaacatacgccgccgacttcaagcggagattcaccttcagcctggacacctccaagagcaccgcctacctccagatgaacagcctgagagccgaggacaccgccgtgtactactgcgccaagtatccctactactacggcaccagccactggtacttcgacgtgtggggacagggcacactggtcacagtgtctagcgcctctacaaagggccccagcgttttcccactggctcctagcagcaagagcacatcaggcggaactgctgccctgggctgtctggtcaaggactactttcctgagcctgtgaccgtgtcctggaacagcggagcactgacatctggcgtgcacacctttccagccgtgctccaaagcagcggcctgtattctctgtccagcgtcgtgacagtgcctagcagctctctgggcacccagacctacatctgcaatgtgaaccacaagcctagcaacaccaaggtcgacaagaaggtggaacccaagagctgcgacaagacccacacctgtcctccatgtcctgctccagaactgctcggcggaccttccgtgttcctgtttcctccaaagcctaaggacaccctgatgatcagcagaacccctgaagtgacctgcgtggtggtggatgtgtcccacgaggatcccgaagtgaagttcaattggtacgtggacggcgtggaagtgcacaacgccaagaccaagcctagagaggaacagtacaatagcacctacagagtggtgtccgtgctgaccgtgctgcaccaggattggctgaacggcaaagagtacaagtgcaaggtgtccaacaaggccctgcctgctcctatcgagaaaaccatctccaaggccaagggccagcctagggaaccccaggtttacacactgcctccaagcagggacgagctgacaaagaaccaggtgtccctgacctgcctggtcaagggcttctacccttccgatatcgccgtggaatgggagagcaatggccagcctgagaacaactacaagacaacccctcctgtgctggacagcgacggctcattcttcctgtacagcaagctgacagtggacaagagcagatggcagcagggcaacgtgttcagctgctccgtgatgcacgaggccctgcacaaccactacacccagaagtccctgagcctgtctcctggcaaatgagccacgcgtaacacgtgcatgcgagagatctga

SEQ ID NO: 73 - protein, 752 aa, Artificial Sequence
  single chain Light-Heavy Ranibizumab fused to Fc
MVLQTQVFISLLLWISGAYGDIQLTQSPSSLSASVGDRVTITCSASQDISNYLNWYQQKPGKAPKVLIYFTSSLHSGVPSRFSGSGSGTDFTLTISSLQPEDFATYYCQQYSTVPWTFGQGTKVEIKRTVAAPSVFIFPPSDEQLKSGTASVVCLLNNFYPREAKVQWKVDNALQSGNSQESVTEQDSKDSTYSLSSTLTLSKADYEKHKVYACEVTHQGLSSPVTKSFNRGECGGSSGSGSGSTGTSSSGTGTSAGTTGTSASTSGSGSGGGGGSGGGGSAGGTATAGASSGSEVQLVESGGGLVQPGGSLRLSCAASGYDFTHYGMNWVRQAPGKGLEWVGWINTYTGEPTYAADFKRRFTFSLDTSKSTAYLQMNSLRAEDTAVYYCAKYPYYYGTSHWYFDVWGQGTLVTVSSASTKGPSVFPLAPSSKSTSGGTAALGCLVKDYFPEPVTVSWNSGALTSGVHTFPAVLQSSGLYSLSSVVTVPSSSLGTQTYICNVNHKPSNTKVDKKVEPKSCDKTHLDKTHTCPPCPAPELLGGPSVFLFPPKPKDTLMISRTPEVTCVVVDVSHEDPEVKFNWYVDGVEVHNAKTKPREEQYNSTYRVVSVLTVLHQDWLNGKEYKCKVSNKALPAPIEKTISKAKGQPREPQVYTLPPSRDELTKNQVSLTCLVKGFYPSDIAVEWESNGQPENNYKTTPPVLDSDGSFFLYSKLTVDKSRWQQGNVFSCSVMHEALHNHYTQKSLSLSPGK

SEQ ID NO: 74 - DNA, 816 bp, Artificial Sequence
  codon optimized Brolucizumab coding sequence
atggtcctccagacacaggtgttcatcagcctgctgctgtggatctctggcgcctatggcgagatcgtgatgacacagagccccagcacactgtctgccagcgtgggagacagagtgatcatcacatgccaggccagcgagatcatccacagctggctggcttggtatcagcagaagcctggcaaggcccctaagctgctgatctacctggcctctacactggccagcggagtgcctagcagattttctggctctggatctggcgccgagttcaccctgacaatctctagcctccagcctgacgacttcgccacctactactgccagaacgtgtacctggccagcaccaacggcgccaattttggccagggcaccaagctgacagtgcttggcggaggcggaggttctggtggcggaggaagtggcggcggaggatcaggcggtggtggatctgaagtgcagctggtggaatcaggcggaggactggttcaacctggcggctctctgagactgagctgtaccgcctctggcttctccctgaccgactactactacatgacctgggtccgacaggcccctggcaaaggacttgagtgggtcggattcatcgaccccgacgacgatccttactacgccacatgggccaagggcagattcaccatcagccgggacaacagcaagaacaccctgtacctccagatgaacagcctgagagccgaggacaccgccgtgtactattgtgccggcggagatcacaatagcggctggggactcgatatctggggccagggaacactggtcaccgtgtctagttga

SEQ ID NO: 75 - protein, 271 aa, Artificial Sequence
  Brolucizumab
MVLQTQVFISLLLWISGAYGEIVMTQSPSTLSASVGDRVIITCQASEIIHSWLAWYQQKPGKAPKLLIYLASTLASGVPSRFSGSGSGAEFTLTISSLQPDDFATYYCQNVYLASTNGANFGQGTKLTVLGGGGGSGGGGSGGGGSGGGGSEVQLVESGGGLVQPGGSLRLSCTASGFSLTDYYYMTWVRQAPGKGLEWVGFIDPDDDPYYATWAKGRFTISRDNSKNTLYLQMNSLRAEDTAVYYCAGGDHNSGWGLDIWGQGTLVTVSS

SEQ ID NO: 76 - DNA, 1530 bp, Artificial Sequence
  Brolucizumab fused to Fc
atggtcctccagacacaggtgttcatcagcctgctgctgtggatctctggcgcctatggcgagatcgtgatgacacagagccccagcacactgtctgccagcgtgggagacagagtgatcatcacatgccaggccagcgagatcatccacagctggctggcttggtatcagcagaagcctggcaaggcccctaagctgctgatctacctggcctctacactggccagcggagtgcctagcagattttctggctctggatctggcgccgagttcaccctgacaatctctagcctccagcctgacgacttcgccacctactactgccagaacgtgtacctggccagcaccaacggcgccaattttggccagggcaccaagctgacagtgcttggcggaggcggaggttctggtggcggaggaagtggcggcggaggatcaggcggtggtggatctgaagtgcagctggtggaatcaggcggaggactggttcaacctggcggctctctgagactgagctgtaccgcctctggcttctccctgaccgactactactacatgacctgggtccgacaggcccctggcaaaggacttgagtgggtcggattcatcgaccccgacgacgatccttactacgccacatgggccaagggcagattcaccatcagccgggacaacagcaagaacaccctgtacctccagatgaacagcctgagagccgaggacaccgccgtgtactattgtgccggcggagatcacaatagcggctggggactcgatatctggggccagggaacactggtcaccgtgtctagtgacaagacccacacctgtcctccatgtcctgctccagaactgctcggcggaccttccgtgttcctgtttcctccaaagcctaaggacaccctgatgatcagcagaacccctgaagtgacctgcgtggtggtggatgtgtcccacgaggatcccgaagtgaagttcaattggtacgtggacggcgtggaagtgcacaacgccaagaccaagcctagagaggaacagtacaatagcacctacagagtggtgtccgtgctgaccgtgctgcaccaggattggctgaacggcaaagagtacaagtgcaaggtgtccaacaaggccctgcctgctcctatcgagaaaaccatctccaaggccaagggccagcctagggaaccccaggtttacacactgcctccaagcagggacgagctgacaaagaaccaggtgtccctgacctgcctggtcaagggcttctacccttccgatatcgccgtggaatgggagagcaatggccagcctgagaacaactacaagacaacccctcctgtgctggacagcgacggctcattcttcctgtacagcaagctgacagtggacaagagcagatggcagcagggcaacgtgttcagctgctccgtgatgcacgaggccctgcacaaccactacacccagaagtccctgagcctgtctcctggcaaatgagccacgcgtaacacgtgcatgcgagagatctga

SEQ ID NO: 77 - protein, 498 aa, Artificial Sequence
  Brolucizumab fused to Fc
MVLQTQVFISLLLWISGAYGEIVMTQSPSTLSASVGDRVIITCQASEIIHSWLAWYQQKPGKAPKLLIYLASTLASGVPSRFSGSGSGAEFTLTISSLQPDDFATYYCQNVYLASTNGANFGQGTKLTVLGGGGGSGGGGSGGGGSGGGGSEVQLVESGGGLVQPGGSLRLSCTASGFSLTDYYYMTWVRQAPGKGLEWVGFIDPDDDPYYATWAKGRFTISRDNSKNTLYLQMNSLRAEDTAVYYCAGGDHNSGWGLDIWGQGTLVTVSSDKTHTCPPCPAPELLGGPSVFLFPPKPKDTLMISRTPEVTCVVVDVSHEDPEVKFNWYVDGVEVHNAKTKPREEQYNSTYRVVSVLTVLHQDWLNGKEYKCKVSNKALPAPIEKTISKAKGQPREPQVYTLPPSRDELTKNQVSLTCLVKGFYPSDIAVEWESNGQPENNYKTTPPVLDSDGSFFLYSKLTVDKSRWQQGNVFSCSVMHEALHNHYTQKSLSLSPGK